European Patent Specification EP 3 442 324 B1, published September 17, 2025. Title: BEGOMOVIRUS-RESISTANT MELON PLANTS. Applicant: Semillas Fito, S.A. The sequence listing filed with the application follows.

SEQUENCE LISTING (56 sequences)

SEQ ID NO: 1 - DNA, 121 bp, Cucumis melo
  variation (61)..(61): T
ttgcaaggtgggctgagatgatgaggaagagggttaagagaagaaatcctacaaactttactaatggtgaccatagcccttagaatctcatttaattaaacaccatttttcacttaatcca

SEQ ID NO: 2 - DNA, 101 bp, Cucumis melo
  variation (51)..(51): C
gtgcatttcatgaaaaaaatagaaactaaaaagtgtgaattttagaaagttcgacttcaaattgaaataaaaaacttaaaatttaaaaaataaaattgtaa

SEQ ID NO: 3 - DNA, 101 bp, Cucumis melo
  variation (51)..(51): T
taaaccaactataacttagggttgtataaattttcaaatgtctgtttcaagggttacttgcataaatgacaaaaaaaaaaaaaaacgtaaaataaaagtat

SEQ ID NO: 4 - DNA, 101 bp, Cucumis melo
  variation (51)..(51): G
cggatgatgtttgtgtctctttgaatttatattaattcactaaatgccatacacacaagttattaatcattaaccaatatcatattatccacggttggaat

SEQ ID NO: 5 - DNA, 101 bp, Cucumis melo
  variation (51)..(51): T
gagagtaattaacacttaggtataattacgacgaataaactacaaaagtagtttgaatttgtgtttttttgagacacaaaggtttttttaaaaatttatat

SEQ ID NO: 6 - DNA, 196 bp, Cucumis melo
  variation (101)..(101): G
gcctatcaggagtgaactcaatctcaatggacatgaaagagaagaagctgacagtaacaggagacgtagatccagtagtgattgtaagcaaattaaggaaaatttgtcatacaacaatagtttccgttggaccagagaaagaagagaagaaaccagaaccaaagaaagatgaaccaaagaaggaagatccaaaaaa

SEQ ID NO: 7 - DNA, 49 bp, Artificial Sequence
  Primer A1 for the detection of SNP Cm_0205
aaggtgaccaagttcatgctgttaagagaagaaatcctacaaactttac

SEQ ID NO: 8 - DNA, 51 bp, Artificial Sequence
  Primer A2 for the detection of SNP CM_0205
gaaggtcggagtcaacggattggttaagagaagaaatcctacaaactttat

SEQ ID NO: 9 - DNA, 26 bp, Artificial Sequence
  Primer C1 for the detection of CM_0205
gagattctaagggctatggtcaccat

SEQ ID NO: 10 - DNA, 54 bp, Artificial Sequence
  Primer A1 for the detection of SNP MEL_SNP_2208
gaaggtgaccaagttcatgctaattttaagttttttatttcaatttgaagtcga

SEQ ID NO: 11 - DNA, 54 bp, Artificial Sequence
  Primer A2 for the detection of SNP MEL_SNP_2208
gaaggtcggagtcaacggattaattttaagttttttatttcaatttgaagtcgg

SEQ ID NO: 12 - DNA, 30 bp, Artificial Sequence
  Primer C1 for the detection of SNP MEL_SNP_2208
agaaactaaaaagtgtgaattttagaaagt

SEQ ID NO: 13 - DNA, 53 bp, Artificial Sequence
  Primer A1 for the detection of SNP MEL_SNP_2224
gaaggtgaccaagttcatgctttttttttttttgtcatttatgcaagtaaccc

SEQ ID NO: 14 - DNA, 52 bp, Artificial Sequence
  Primer A2 for the detection of SNP MEL_SNP_2224
gaaggtcggagtcaacggatttttttttttttgtcatttatgcaagtaacca

SEQ ID NO: 15 - DNA, 30 bp, Artificial Sequence
  Primer C1 for the detection of SNP MEL_SNP_2224
agggttgtataaattttcaaatgtctgttt

SEQ ID NO: 16 - DNA, 52 bp, Artificial Sequence
  Primer A1 for the detection of SNP MEL_SNP_4105
gaaggtgaccaagttcatgctttgaatttatattaattcactaaatgccata

SEQ ID NO: 17 - DNA, 54 bp, Artificial Sequence
  Primer A2 for the detection of SNP MEL_SNP_4105
gaaggtcggagtcaacggattgagagtatattttaaatttttaataaaacattg

SEQ ID NO: 18 - DNA, 30 bp, Artificial Sequence
  Primer C1 for the detection of SNP MEL_SNP_4105
cattttttagagtagtagtgagcatgtcaa

SEQ ID NO: 19 - DNA, 53 bp, Artificial Sequence
  Primer A1 for the detection of SNP MEL_SNP_4114
gaaggtgaccaagttcatgctgtataattacgacgaataaactacaaaagtag

SEQ ID NO: 20 - DNA, 53 bp, Artificial Sequence
  Primer A2 for the detection of SNP MEL_SNP_4114
gaaggtcggagtcaacggattgtataattacgacgaataaactacaaaagtat

SEQ ID NO: 21 - DNA, 30 bp, Artificial Sequence
  Primer C1 for the detection of SNP MEL_SNP_4114
cctttgtgtctcaaaaaaacacaaattcaa

SEQ ID NO: 22 - DNA, 50 bp, Artificial Sequence
  Primer A1 for the detection of SNP SFMe066
gaaggtgaccaagttcatgctcagtagtgattgtaagcaaattaaggaaa

SEQ ID NO: 23 - DNA, 50 bp, Artificial Sequence
  Primer A2 for the detection of SNP SFMe066
gaaggtcggagtcaacggattcagtagtgattgtaagcaaattaaggaag

SEQ ID NO: 24 - DNA, 29 bp, Artificial Sequence
  Primer C1 for the detection of SNP SFMe066
gtccaacggaaactattgttgtatgacaa

SEQ ID NO: 25 - DNA, 101 bp, Cucumis melo
  variation (51)..(51): A
gtaatagaactcggcaatggtttcttttcaactctatttcctaaaggcagtaaatatttgattgattgcatcttaacagttagaggtataaacatgttttc

SEQ ID NO: 26 - DNA, 101 bp, Cucumis melo
  variation (51)..(51): A
tgaaaactcatcctttttccacagaatctgtattacaaggcaaaaaagaagaagctacatatcaaatattatatctaaaaatggagatccatgtactacca

SEQ ID NO: 27 - DNA, 101 bp, Cucumis melo
  variation (51)..(51): C
aaaaactcccaaatggagtacacaatttgttttaaaaaaaccaaaggttatgaatcaatttaattccttaaaacctttaaattctattaataatatgaaac

SEQ ID NO: 28 - DNA, 101 bp, Cucumis melo
  variation (51)..(51): C
agtctagacttttttataacatttttccaaaactatagtggatgctataatagtgtatgaatgtaatacgttgctatataaaaactttttatagtgttttt

SEQ ID NO: 29 - DNA, 101 bp, Cucumis melo
  variation (51)..(51): A
ggaagagaaaagcctccttcatagagttttaaaacatcttgaaaagagtcgaactctcctggatttctgctaaataattcatcaagggctggtttaataga

SEQ ID NO: 30 - DNA, 101 bp, Cucumis melo
  variation (51)..(51): C
attgaattgaatccatttgaatttttaaaagtgtatcccggacctaattatccaagattaatacttgtttttaaatgcactttaccgttttgttaaaagaa

SEQ ID NO: 31 - DNA, 101 bp, Cucumis melo
  variation (51)..(51): A
aaacttacagcttccaagttgagacaatcattctcaccttcaagattggctgctaggttggtgtctcccctgaaaagcagaaaaagtgtacaaaagtatga

SEQ ID NO: 32 - DNA, 101 bp, Cucumis melo
  variation (51)..(51): C
ttacaagtgagatttgcattttttagagtagtagtgagcatgtcaaatgtgaatgttttattaaaaatttaaaatatactctctttaacaaaaaattaaga

SEQ ID NO: 33 - DNA, 47 bp, Artificial Sequence
  Primer A1 for the detection of SNP CM_5_1
gaaggtgaccaagttcatgcttttcaactctatttcctaaaggcagt

SEQ ID NO: 34 - DNA, 49 bp, Artificial Sequence
  Primer A2 for the detection of SNP CM_5_1
gaaggtcggagtcaacggattcttttcaactctatttcctaaaggcaga

SEQ ID NO: 35 - DNA, 30 bp, Artificial Sequence
  Primer C1 for the detection of SNP CM_5_1
cctctaactgttaagatgcaatcaatcaaa

SEQ ID NO: 36 - DNA, 50 bp, Artificial Sequence
  Primer A1 for the detection of SNP CM_5_2
gaaggtgaccaagttcatgctagaatctgtattacaaggcaaaaaagaag

SEQ ID NO: 37 - DNA, 51 bp, Artificial Sequence
  Primer A2 for the detection of SNP CM_5_2
gaaggtcggagtcaacggattcagaatctgtattacaaggcaaaaaagaaa

SEQ ID NO: 38 - DNA, 30 bp, Artificial Sequence
  Primer C1 for the detection of SNP CM_5_2
ggtagtacatggatctccatttttagatat

SEQ ID NO: 39 - DNA, 54 bp, Artificial Sequence
  rimer A1 for the detection of SNP CM_5_3
gaaggtgaccaagttcatgctaatttaaaggttttaaggaattaaattgattca

SEQ ID NO: 40 - DNA, 54 bp, Artificial Sequence
  Primer A2 for the detection of SNP CM_5_3
gaaggtcggagtcaacggattaatttaaaggttttaaggaattaaattgattcg

SEQ ID NO: 41 - DNA, 30 bp, Artificial Sequence
  Primer C1 for the detection of SNP CM_5_3
aaactcccaaatggagtacacaatttgttt

SEQ ID NO: 42 - DNA, 53 bp, Artificial Sequence
  Primer A1 for the detection of SNP CM_5_4
gaaggtgaccaagttcatgcttttatatagcaacgtattacattcatacacta

SEQ ID NO: 43 - DNA, 50 bp, Artificial Sequence
  Primer A2 for the detection of SNP CM_5_4
gaaggtcggagtcaacggattatatagcaacgtattacattcatacactg

SEQ ID NO: 44 - DNA, 30 bp, Artificial Sequence
  Primer C1 for the detection of SNP CM_5_4
catttttccaaaactatagtggatgctata

SEQ ID NO: 45 - DNA, 47 bp, Artificial Sequence
  Primer A1 for the detection of SNP CM_5_5
gaaggtgaccaagttcatgcttatttagcagaaatccaggagagttc

SEQ ID NO: 46 - DNA, 50 bp, Artificial Sequence
  Primer A2 for the detection of SNP CM_5_5
gaaggtcggagtcaacggattaattatttagcagaaatccaggagagttt

SEQ ID NO: 47 - DNA, 30 bp, Artificial Sequence
  Primer C1 for the detection of SNP CM_5_5
agcctccttcatagagttttaaaacatctt

SEQ ID NO: 48 - DNA, 54 bp, Artificial Sequence
  Primer A1 for the detection of SNP CM_5_6
gaaggtgaccaagttcatgctaaagtgcatttaaaaacaagtattaatcttgga

SEQ ID NO: 49 - DNA, 51 bp, Artificial Sequence
  Primer A2 for the detection of SNP CM_5_6
gaaggtcggagtcaacggattgtgcatttaaaaacaagtattaatcttggg

SEQ ID NO: 50 - DNA, 30 bp, Artificial Sequence
  Primer C1 for the detection of SNP CM_5_6
gaatttttaaaagtgtatcccggacctaat

SEQ ID NO: 51 - DNA, 47 bp, Artificial Sequence
  Primer A1 for the detection of SNP CM_5_7
gaaggtgaccaagttcatgctaatcattctcaccttcaagattggct

SEQ ID NO: 52 - DNA, 47 bp, Artificial Sequence
  Primer A2 for the detection of SNP CM_5_7
gaaggtcggagtcaacggattaatcattctcaccttcaagattggca

SEQ ID NO: 53 - DNA, 25 bp, Artificial Sequence
  Primer C1 for the detection of SNP CM_5_7
ttctgcttttcaggggagacaccaa

SEQ ID NO: 54 - DNA, 54 bp, Artificial Sequence
  Primer A1 for the detection of SNP CM_9_1
gaaggtgaccaagttcatgctgagagtatattttaaatttttaataaaacattc

SEQ ID NO: 55 - DNA, 54 bp, Artificial Sequence
  Primer A2 for the detection of SNP CM_9_1
gaaggtcggagtcaacggattctttgaatttatattaattcactaaatgccatg

SEQ ID NO: 56 - DNA, 30 bp, Artificial Sequence
  Primer C1 for the detection of SNP CM_9_1
ccaaccgtggataatatgatattggttaat